European Patent Application EP 4 678 768 A1, published January 14, 2026. Title: SIGNATURE FOR PROGNOSIS OF METASTASIS RISK AND CHEMOTHERAPY RESPONSE. Applicant: Fundación de la Comunidad Valenciana Centro de Investigación Príncipe Felipe. The sequence listing filed with the application follows.

SEQUENCE LISTING (12 sequences)

SEQ ID NO: 1 - DNA, 22 bp, synthetic construct
  source 1..22: mol_type = other DNA; note = Forward primer for gene HAS2; note (original language) = Cebador directo para el gen HAS2
ctcttttggactgtatggtgcc

SEQ ID NO: 2 - DNA, 22 bp, synthetic construct
  source 1..22: mol_type = other DNA; note = Reverse primer for HAS2 gene; note (original language) = Cebador inverso para el gen HAS2
agggtaggttagccttttcaca

SEQ ID NO: 3 - DNA, 21 bp, synthetic construct
  source 1..21: mol_type = other DNA; note = Forward Primer for gene HPRT; note (original language) = Cebador directo para el gen HPRT
cctggcgtcgtgattagtgat

SEQ ID NO: 4 - DNA, 22 bp, synthetic construct
  source 1..22: mol_type = other DNA; note = Reverse primer for HPRT gene; note (original language) = Cebador inverso para el gen HPRT
agacgttcagtcctgtccataa

SEQ ID NO: 5 - DNA, 22 bp, synthetic construct
  source 1..22: mol_type = other DNA; note = Forward primer for gene HAPLN1; note (original language) = Cebador directo para el gen HAPLN1
tctggtgctgatttcaatctgc

SEQ ID NO: 6 - DNA, 22 bp, synthetic construct
  source 1..22: mol_type = other DNA; note = Reverse primer for gene HAPLN1; note (original language) = Cebador inverso para el gen HAPLN1
tctggtgctgatttcaatctgc

SEQ ID NO: 7 - DNA, 23 bp, synthetic construct
  source 1..23: mol_type = other DNA; note = Forward primer for gene TNFAIP6; note (original language) = Cebador directo para el gen TNFAIP6
tttctcttgctatgggaagacac

SEQ ID NO: 8 - DNA, 21 bp, synthetic construct
  source 1..21: mol_type = other DNA; note = Reverse primer for gene TNFAIP6; note (original language) = Cebador inverso para el gen TNFAIP6
gagcttgtatttgccagaccg

SEQ ID NO: 9 - DNA, 21 bp, synthetic construct
  source 1..21: mol_type = other DNA; note = Forward primer for gene TNFRSF1B; note (original language) = Cebador directo para el gen TNFRSF1B
tgaaacatcagacgtggtgtg

SEQ ID NO: 10 - DNA, 23 bp, synthetic construct
  source 1..23: mol_type = other DNA; note = Reverse primer for gene TNFRSF1B; note (original language) = Cebador inverso para el gen TNFRSF1B
tgcaaatatccgtggatgaagtc

SEQ ID NO: 11 - DNA, 27 bp, synthetic construct
  source 1..27: mol_type = other DNA; note = Forward PCR primer for analysing micoplasma contamination; note (original language) = Cebador directo de PCR para analizar contaminación con micoplasmas
gggagcaaacaggattagatataccct

SEQ ID NO: 12 - DNA, 31 bp, synthetic construct
  source 1..31: mol_type = other DNA; note = Reverse PCR primer for analysing micoplasm contamination; note (original language) = Cebador inverso de PCR para analizar contaminación con micoplasmas
tcggaccatcatctgtcactctgttaacctc